European Patent Application EP 4 417 619 A1, published August 21, 2024. Title: NUCLEOTIDE SEQUENCE ENCODING A FUSED PROTEIN CONSISTING OF A SOLUBLE EXTRACELLULAR FRAGMENT OF HUMAN Dll4 AND THE CONSTANT PART OF THE HEAVY CHAIN OF HUMAN IgG4. Applicant: Palmira Biopharma Limited Liability Company / "PALMIRA BIOPHARMA" Limited Liability Company. The sequence listing filed with the application follows.

SEQUENCE LISTING (22 sequences)

SEQ ID NO: 1 - protein, 685 aa, Homo sapiens
MAAASRSASGWALLLLVALWQQRAAGSGVFQLQLQEFINERGVLASGRPCEPGCRTFFRVCLKHFQAVVSPGPCTFGTVSTPVLGTNSFAVRDDSSGGGRNPLQLPFNFTWPGTFSLIIEAWHAPGDDLRPEALPPDALISKIAIQGSLAVGQNWLLDEQTSTLTRLRYSYRVICSDNYYGDNCSRLCKKRNDHFGHYVCQPDGNLSCLPGWTGEYCQQPICLSGCHEQNGYCSKPAECLCRPGWQGRLCNECIPHNGCRHGTCSTPWQCTCDEGWGGLFCDQDLNYCTHHSPCKNGATCSNSGQRSYTCTCRPGYTGVDCELELSECDSNPCRNGGSCKDQEDGYHCLCPPGYYGLHCEHSTLSCADSPCFNGGSCRERNQGANYACECPPNFTGSNCEKKVDRCTSNPCANGGQCLNRGPSRMCRCRPGFTGTYCELHVSDCARNPCAHGGTCHDLENGLMCTCPAGFSGRRCEVRTSIDACASSPCFNRATCYTDLSTDTFVCNCPYGFVGSRCEFPVGLPPSFPWVAVSLGVGLAVLLVLLGMVAVAVRQLRLRRPDDGSREAMNNLSDFQKDNLIPAAQLKNTNQKKELEVDCGLDKSNCGKQQNHTLDYNLAPGPLGRGTMPGKFPHSDKSLGEKAPLRLHSEKPECRISAICSPRDSMYQSVCLISEERNECVIATEV

SEQ ID NO: 2 - protein, 482 aa, artificial sequence
  hybrid protein
MYRMQLLSCIALSLALVTNSYRVICSDNYYGDNCSRLCKKRNDHFGHYVCQPDGNLSCLPGWTGEYCQQPICLSGCHEQNGYCSKPAECLCRPGWQGRLCNECIPHNGCRHGTCSTPWQCTCDEGWGGLFCDQDLNYCTHHSPCKNGATCSNSGQRSYTCTCRPGYTGVDCELELSECDSNPCRNGGSCKDQEDGYHCLCPPGYYGLHCEHSTLSCADSPCFNGGSCRERNQGANYACECPPNFTGSNCEKKVDGSYGPPCPPCPAPEFLGGPSVFLFPPKPKDTLMISRTPEVTCVVVDVSQEDPEVQFNWYVDGVEVHNAKTKPREEQFNSTYRVVSVLTVLHQDWLNGKEYKCKVSNKGLPSSIEKTISKAKGQPREPQVYTLPPSQEEMTKNQVSLTCLVKGFYPSDIAVEWESNGQPENNYKTTPPVLDSDGSFFLYSRLTVDKSRWQEGNVFSCSVMHEALHNHYTQKSLSLSPGK

SEQ ID NO: 3 - DNA, 1446 bp, artificial sequence
  nucleotide sequence encoding hybrid protein
atgtacaggatgcaactcctgtcttgcattgcactaagtcttgcacttgtcacgaattcctaccgggtcatctgcagtgacaactactatggagacaactgctcccgcctgtgcaagaagcgcaatgaccacttcggccactatgtgtgccagccagatggcaacttgtcctgcctgcccggttggactggggaatattgccaacagcctatctgtctttcgggctgtcatgaacagaatggctactgcagcaagccagcagagtgcctctgccgcccaggctggcagggccggctgtgtaacgaatgcatcccccacaatggctgtcgccacggcacctgcagcactccctggcaatgtacttgtgatgagggctggggaggcctgttttgtgaccaagatctcaactactgcacccaccactccccatgcaagaatggggcaacgtgctccaacagtgggcagcgaagctacacctgcacctgtcgcccaggctacactggtgtggactgtgagctggagctcagcgagtgtgacagcaacccctgtcgcaatggaggcagctgtaaggaccaggaggatggctaccactgcctgtgtcctccgggctactatggcctgcattgtgaacacagcaccttgagctgcgccgactccccctgcttcaatgggggctcctgccgggagcgcaaccagggggccaactatgcttgtgaatgtccccccaacttcaccggctccaactgcgagaagaaagtggacggatcttatggtcccccatgcccaccatgcccagcacctgagttcctggggggaccatcagtcttcctgttccccccaaaacccaaggacactctcatgatctcccggacccctgaggtcacgtgcgtggtggtggacgtgagccaggaagaccccgaggtccagttcaactggtacgtggatggcgtggaggtgcataatgccaagacaaagccgcgggaggagcagttcaacagcacgtaccgtgtggtcagcgtcctcaccgtcctgcaccaggactggctgaacggcaaggagtacaagtgcaaggtctccaacaaaggcctcccgtcctccatcgagaaaaccatctccaaagccaaagggcagccccgagagccacaggtgtacaccctgcccccatcccaggaggagatgaccaagaaccaggtcagcctgacctgcctggtcaaaggcttctaccccagcgacatcgccgtggagtgggagagcaatgggcagccggagaacaactacaagaccacgcctcccgtgctggactccgacggctccttcttcctctacagcaggctaaccgtggacaagagcaggtggcaggaggggaatgtcttctcatgctccgtgatgcatgaggctctgcacaaccactacacacagaagagcctctccctgtctccgggtaaa

SEQ ID NO: 4 - protein, 593 aa, artificial sequence
  hybrid protein
MYRMQLLSCIALSLALVTNSYRVICSDNYYGDNCSRLCKKRNDHFGHYVCQPDGNLSCLPGWTGEYCQQPICLSGCHEQNGYCSKPAECLCRPGWQGRLCNECIPHNGCRHGTCSTPWQCTCDEGWGGLFCDQDLNYCTHHSPCKNGATCSNSGQRSYTCTCRPGYTGVDCELELSECDSNPCRNGGSCKDQEDGYHCLCPPGYYGLHCEHSTLSCADSPCFNGGSCRERNQGANYACECPPNFTGSNCEKKVDRCTSNPCANGGQCLNRGPSRMCRCRPGFTGTYCELHVSDCARNPCAHGGTCHDLENGLMCTCPAGFSGRRCEVRTSIDACASSPCFNRATCYTDLSTDTFVCNCPYGFVGSGSYGPPCPPCPAPEFLGGPSVFLFPPKPKDTLMISRTPEVTCVVVDVSQEDPEVQFNWYVDGVEVHNAKTKPREEQFNSTYRVVSVLTVLHQDWLNGKEYKCKVSNKGLPSSIEKTISKAKGQPREPQVYTLPPSQEEMTKNQVSLTCLVKGFYPSDIAVEWESNGQPENNYKTTPPVLDSDGSFFLYSRLTVDKSRWQEGNVFSCSVMHEALHNHYTQKSLSLSPGK

SEQ ID NO: 5 - DNA, 1779 bp, artificial sequence
  nucleotide sequence encoding hybrid protein
atgtacaggatgcaactcctgtcttgcattgcactaagtcttgcacttgtcacgaattcctaccgggtcatctgcagtgacaactactatggagacaactgctcccgcctgtgcaagaagcgcaatgaccacttcggccactatgtgtgccagccagatggcaacttgtcctgcctgcccggttggactggggaatattgccaacagcctatctgtctttcgggctgtcatgaacagaatggctactgcagcaagccagcagagtgcctctgccgcccaggctggcagggccggctgtgtaacgaatgcatcccccacaatggctgtcgccacggcacctgcagcactccctggcaatgtacttgtgatgagggctggggaggcctgttttgtgaccaagatctcaactactgcacccaccactccccatgcaagaatggggcaacgtgctccaacagtgggcagcgaagctacacctgcacctgtcgcccaggctacactggtgtggactgtgagctggagctcagcgagtgtgacagcaacccctgtcgcaatggaggcagctgtaaggaccaggaggatggctaccactgcctgtgtcctccgggctactatggcctgcattgtgaacacagcaccttgagctgcgccgactccccctgcttcaatgggggctcctgccgggagcgcaaccagggggccaactatgcttgtgaatgtccccccaacttcaccggctccaactgcgagaagaaagtggacaggtgcaccagcaacccctgtgccaacgggggacagtgcctgaaccgaggtccaagccgcatgtgccgctgccgtcctggattcacgggcacctactgtgaactccacgtcagcgactgtgcccgtaacccttgcgcccacggtggcacttgccatgacctggagaatgggctcatgtgcacctgccctgccggcttctctggccgacgctgtgaggtgcggacatccatcgatgcctgtgcctcgagtccctgcttcaacagggccacctgctacaccgacctctccacagacacctttgtgtgcaactgcccttatggctttgtgggcagcggatcttatggtcccccatgcccaccatgcccagcacctgagttcctggggggaccatcagtcttcctgttccccccaaaacccaaggacactctcatgatctcccggacccctgaggtcacgtgcgtggtggtggacgtgagccaggaagaccccgaggtccagttcaactggtacgtggatggcgtggaggtgcataatgccaagacaaagccgcgggaggagcagttcaacagcacgtaccgtgtggtcagcgtcctcaccgtcctgcaccaggactggctgaacggcaaggagtacaagtgcaaggtctccaacaaaggcctcccgtcctccatcgagaaaaccatctccaaagccaaagggcagccccgagagccacaggtgtacaccctgcccccatcccaggaggagatgaccaagaaccaggtcagcctgacctgcctggtcaaaggcttctaccccagcgacatcgccgtggagtgggagagcaatgggcagccggagaacaactacaagaccacgcctcccgtgctggactccgacggctccttcttcctctacagcaggctaaccgtggacaagagcaggtggcaggaggggaatgtcttctcatgctccgtgatgcatgaggctctgcacaaccactacacacagaagagcctctccctgtctccgggtaaa

SEQ ID NO: 6 - protein, 234 aa, Homo sapiens
  protein fragment
YRVICSDNYYGDNCSRLCKKRNDHFGHYVCQPDGNLSCLPGWTGEYCQQPICLSGCHEQNGYCSKPAECLCRPGWQGRLCNECIPHNGCRHGTCSTPWQCTCDEGWGGLFCDQDLNYCTHHSPCKNGATCSNSGQRSYTCTCRPGYTGVDCELELSECDSNPCRNGGSCKDQEDGYHCLCPPGYYGLHCEHSTLSCADSPCFNGGSCRERNQGANYACECPPNFTGSNCEKKVD

SEQ ID NO: 7 - protein, 226 aa, Homo sapiens
  Fc region of IgG4
YGPPCPPCPAPEFLGGPSVFLFPPKPKDTLMISRTPEVTCVVVDVSQEDPEVQFNWYVDGVEVHNAKTKPREEQFNSTYRVVSVLTVLHQDWLNGKEYKCKVSNKGLPSSIEKTISKAKGQPREPQVYTLPPSQEEMTKNQVSLTCLVKGFYPSDIAVEWESNGQPENNYKTTPPVLDSDGSFFLYSRLTVDKSRWQEGNVFSCSVMHEALHNHYTQKSLSLSPGK

SEQ ID NO: 8 - DNA, 35 bp, artificial sequence
  primer
aagaattcctaccgggtcatctgcagtgacaacta

SEQ ID NO: 9 - DNA, 32 bp, artificial sequence
  primer
taggatccgtccactttcttctcgcagttgga

SEQ ID NO: 10 - DNA, 32 bp, artificial sequence
  primer
taggatccgctgcccacaaagccataagggca

SEQ ID NO: 11 - DNA, 22 bp, artificial sequence
  primer
gcctgaccctgcttgctcaact

SEQ ID NO: 12 - DNA, 20 bp, artificial sequence
  primer
ctcacgtccaccaccacgca

SEQ ID NO: 13 - DNA, 20 bp, artificial sequence
  primer
aagaaagatagctcgcggca

SEQ ID NO: 14 - DNA, 20 bp, artificial sequence
  primer
tacttccccagcacacttgg

SEQ ID NO: 15 - DNA, 22 bp, artificial sequence
  primer
gattcctctgtgtgggtggatg

SEQ ID NO: 16 - DNA, 22 bp, artificial sequence
  primer
gattttattatggcggcttcgg

SEQ ID NO: 17 - DNA, 20 bp, artificial sequence
  primer
ccttccccttctctttcggc

SEQ ID NO: 18 - DNA, 20 bp, artificial sequence
  primer
aaaagctccgatctccgtcc

SEQ ID NO: 19 - DNA, 20 bp, artificial sequence
  primer
aaggcgtcgggatcggataa

SEQ ID NO: 20 - DNA, 21 bp, artificial sequence
  primer
agagcgtgtgcgtcaaagtag

SEQ ID NO: 21 - DNA, 20 bp, artificial sequence
  primer
ccatcaccatcttccaggag

SEQ ID NO: 22 - DNA, 20 bp, artificial sequence
  primer
aatgagccccagccttctcc